European Patent Application EP 4 269 564 A1, published November 1, 2023. Title: CHEMICAL INDUCTION METHOD FOR PHOTORECEPTOR NEURON CELLS. Applicant: REGENE THERAPEUTICS LTD. The sequence listing filed with the application follows.

SEQUENCE LISTING (22 sequences)

SEQ ID NO: 1 - DNA, 21 bp, Artificial Sequence
  SOX2-F
catgcaggttgacaccgttgg

SEQ ID NO: 2 - DNA, 24 bp, Artificial Sequence
  SOX2-R
atggattctcggcagactgattca

SEQ ID NO: 3 - DNA, 19 bp, Artificial Sequence
  PAX6-F
tctttgcttgggaaatccg

SEQ ID NO: 4 - DNA, 21 bp, Artificial Sequence
  PAX6-R
ctgcccgttcaacatccttag

SEQ ID NO: 5 - DNA, 23 bp, Artificial Sequence
  CASP3-F
ggaagcgaatcaatggactctgg

SEQ ID NO: 6 - DNA, 22 bp, Artificial Sequence
  CASP3-R
gcatcgacatctgtaccagacc

SEQ ID NO: 7 - DNA, 20 bp, Artificial Sequence
  ACTIN-F
tccctggagaagagctacga

SEQ ID NO: 8 - DNA, 20 bp, Artificial Sequence
  ACTIN-R
agcactgtgttggcgtacag

SEQ ID NO: 9 - DNA, 22 bp, Artificial Sequence
  Nestin-F
tcaagatgtccctcagcctgga

SEQ ID NO: 10 - DNA, 23 bp, Artificial Sequence
  Nestin-R
tggcacaggtgtctcaagggtag

SEQ ID NO: 11 - DNA, 25 bp, Artificial Sequence
  CRX-F
cttgtagaggacgcagtctccatct

SEQ ID NO: 12 - DNA, 23 bp, Artificial Sequence
  CRX-R
caatcgtgccagacggtgttagg

SEQ ID NO: 13 - DNA, 24 bp, Artificial Sequence
  OPN1LW-F
tcatcgccagcactatcagcattg

SEQ ID NO: 14 - DNA, 24 bp, Artificial Sequence
  OPN1LW-R
acagcagaccagatccaggagaag

SEQ ID NO: 15 - DNA, 24 bp, Artificial Sequence
  Recoverin-F
cagttccagagcatctacgccaag

SEQ ID NO: 16 - DNA, 23 bp, Artificial Sequence
  Recoverin-R
gccatgacgatctccagcacttc

SEQ ID NO: 17 - DNA, 24 bp, Artificial Sequence
  Rhodopsin-F
cagcgtggcattctacatcttcac

SEQ ID NO: 18 - DNA, 20 bp, Artificial Sequence
  Rhodopsin-R
acctggctcgtctccgtctt

SEQ ID NO: 19 - DNA, 19 bp, Artificial Sequence
  PAX6-F
tctttgcttgggaaatccg

SEQ ID NO: 20 - DNA, 21 bp, Artificial Sequence
  PAX6-R
ctgcccgttcaacatccttag

SEQ ID NO: 21 - DNA, 22 bp, Artificial Sequence
  βActin-F
ggccgaggactttgattgcaca

SEQ ID NO: 22 - DNA, 23 bp, Artificial Sequence
  βActin-R
gggcacgaaggctcatcattcaa